European Patent Specification EP 3 795 696 B1, published April 26, 2023. Title: IDENTIFICATION AND USE OF CIRCULATING NUCLEIC ACID TUMOR MARKERS. Applicant: THE BOARD OF TRUSTEES OF THE LELAND STANFORD JUNIOR UNIVERSITY. The sequence listing filed with the application follows.

SEQUENCE LISTING (32 sequences)

SEQ ID NO: 1 - DNA, 101 bp, Homo sapiens
agaaatactaataaaatgattaaagaaggtgtgtctttaattgaagcatgatttaaagtaaatgcaaagctaaaaatcagaccactgcactccagcctggg

SEQ ID NO: 2 - DNA, 101 bp, Homo sapiens
tactaataaaatgattaaagaaggtgtgtctttaattgaagcatgatttaaagtaaatgcaaagctaaaaatcagaccactgcactccagcctggggaaca

SEQ ID NO: 3 - DNA, 101 bp, Homo sapiens
aaatgattaaagaaggtgtgtctttaattgaagcatgatttaaagtaaatgcaaagctaaaaatcagaccactgcactccagcctggggaacaagagtgaa

SEQ ID NO: 4 - DNA, 101 bp, Homo sapiens
gtgtgtctttaattgaagcatgatttaaagtaaatgcaaagctaaaaatcagaccactgcactccagcctggggaacaagagtgaaaccccatctcaaaaa

SEQ ID NO: 5 - DNA, 100 bp, Homo sapiens
gtgtctttaattgaagcatgatttaaagtaaatgcaaagctaaaaatcagaccactgcactccagcctggggaacaagagtgaaaccccatctcaaaaac

SEQ ID NO: 6 - DNA, 100 bp, Homo sapiens
gtctttaattgaagcatgatttaaagtaaatgcaaagctaaaaatcagaccactgcactccagcctggggaacaagagtgaaaccccatctcaaaaacaa

SEQ ID NO: 7 - DNA, 92 bp, Homo sapiens
tgaagcatgatttaaagtaaatgcaaagctaaaaatcagaccactgcactccagcctggggaacaagagtgaaaccccatctcaaaaacaaa

SEQ ID NO: 8 - DNA, 92 bp, Homo sapiens
atgatttaaagtaaatgcaaagctaaaaatcagaccactgcactccagcctggggaacaagagtgaaaccccatctcaaaaacaaacaaaca

SEQ ID NO: 9 - DNA, 92 bp, Homo sapiens
agtaaatgcaaagctaaaaatcagaccactgcactccagcctggggaacaagagtgaaaccccatctcaaaaacaaacaaacaaaacaaaac

SEQ ID NO: 10 - DNA, 100 bp, Homo sapiens
atgcaaagctaaaaatcagaccactgcactccagcctggggaacaagagtgaaaccccatctcaaaaacaaacaaacaaaacaaaacaaaaaaaactaag

SEQ ID NO: 11 - DNA, 40 bp, Homo sapiens
atgcaaagctaaaaatcagaccactgcactccagcctggg

SEQ ID NO: 12 - DNA, 101 bp, Homo sapiens
tgtcagagtagtggtggtttataagacgggagaaaatagcacctcacttccagaaagctttaagacaaaaggtgagtactagagtaagattcagtctcaga

SEQ ID NO: 13 - DNA, 101 bp, Homo sapiens
gagtagtggtggtttataagacgggagaaaatagcacctcacttccagaaagctttaagacaaaaggtgagtactagagtaagattcagtctcagatctgg

SEQ ID NO: 14 - DNA, 103 bp, Homo sapiens
gtggtggtttataagacgggagaaaatagcacctcacttccagaaagctttaagacaaaaggtgagtactagagtaagattcagtctcagatctgggtgacac

SEQ ID NO: 15 - DNA, 101 bp, Homo sapiens
gtttataagacgggagaaaatagcacctcacttccagaaagctttaagacaaaaggtgagtactagagtaagattcagtctcagatctgggtgacacaaag

SEQ ID NO: 16 - DNA, 101 bp, Homo sapiens
ataagacgggagaaaatagcacctcacttccagaaagctttaagacaaaaggtgagtactagagtaagattcagtctcagatctgggtgacacaaaggacc

SEQ ID NO: 17 - DNA, 101 bp, Homo sapiens
agaaaatagcacctcacttccagaaagctttaagacaaaaggtgagtactagagtaagattcagtctcagatctgggtgacacaaaggaccatggatttct

SEQ ID NO: 18 - DNA, 101 bp, Homo sapiens
aatagcacctcacttccagaaagctttaagacaaaaggtgagtactagagtaagattcagtctcagatctgggtgacacaaaggaccatggatttctgcaa

SEQ ID NO: 19 - DNA, 104 bp, Homo sapiens
acctcacttccagaaagctttaagacaaaaggtgagtactagagtaagattcagtctcagatctgggtgacacaaaggaccatggatttctgcaacccttggtg

SEQ ID NO: 20 - DNA, 101 bp, Homo sapiens
cagaaagctttaagacaaaaggtgagtactagagtaagattcagtctcagatctgggtgacacaaaggaccatggatttctgcaacccttggtgcctttct

SEQ ID NO: 21 - DNA, 101 bp, Homo sapiens
aagacaaaaggtgagtactagagtaagattcagtctcagatctgggtgacacaaaggaccatggatttctgcaacccttggtgcctttcttgggaacccat

SEQ ID NO: 22 - DNA, 40 bp, Homo sapiens
aagacaaaaggtgagtactagagtaagattcagtctcaga

SEQ ID NO: 23 - DNA, 20 bp, Artificial sequence
  synthetic polynucleotide
agacgggagaaaatagcacc

SEQ ID NO: 24 - DNA, 20 bp, Artificial sequence
  synthetic polynucleotide
accaagggttgcagaaatcc

SEQ ID NO: 25 - DNA, 24 bp, Artificial sequence
  synthetic polynucleotide
gagatggagtttcactcttgttgc

SEQ ID NO: 26 - DNA, 27 bp, Artificial sequence
  synthetic polynucleotide
gaacctttccatcatacttagaaatac

SEQ ID NO: 27 - DNA, 17 bp, Artificial sequence
  synthetic polynucleotide
tccatggaagccagaac

SEQ ID NO: 28 - DNA, 20 bp, Artificial sequence
  synthetic polynucleotide
atgctaagatgtgtctgtca

SEQ ID NO: 29 - DNA, 25 bp, Artificial sequence
  synthetic polynucleotide
ccttaacacagatggctcttgatgc

SEQ ID NO: 30 - DNA, 23 bp, Artificial sequence
  synthetic polynucleotide
tcctctttccaccttggctttcc

SEQ ID NO: 31 - DNA, 23 bp, Artificial sequence
  synthetic polynucleotide
ggttcagaactaccaataacaag

SEQ ID NO: 32 - DNA, 24 bp, Artificial Sequence
  synthetic polynucleotide
acctgatgtgtgacctgattgatg